European Patent Specification EP 3 682 907 B1, published April 23, 2025. Title: USE OF RADIOLABELED ANTI-NANOBODY IN PROGNOSIS AND DIAGNOSIS OF CANCER. Applicant: NANOMAB TECHNOLOGY LIMITED. The sequence listing filed with the application follows.

SEQUENCE LISTING (3 sequences)

SEQ ID NO: 1 - protein, 127 aa, Artificial Sequence
  VHH chain
QVQLQESGGGSVQTGGSLRLSCAASTSIYSNNYMAWFSQAPGKGREGVAAVYIDDGRPYYADSVKGRFTISLDSAKNTVYLQMNRLKPEDTAMYYCAAAPGPLSHNYWYTSANYDYWGQGTQVTVSS

SEQ ID NO: 2 - protein, 124 aa, Artificial Sequence
  VHH chain
QVQLQESGGGSVQAGGSLRLSCAASGYTYSSDGMGWFRQTPGKEREGVAAISPTGRRTEYADSVKGRFTISRDNNKNMLSLQMNSLKPEDTGMYYCAREGSWSFSLANSAVRSWGQGTQVTVSS

SEQ ID NO: 3 - protein, 127 aa, Artificial Sequence
  VHH chain
QVQLQESGGGSVQTGGSLRLSCTASTSIYSNNYMAWFSQSPGKGREGVAAVYMDDGRPYYADSVKGRFTISLDSAKNTMYLQMNSLKPEDTAMYYCAAAPGPLSRNYWYTSANYDYWGQGTQVTVSS